European Patent Application EP 4 483 895 A2, published January 1, 2025. Title: Antibodies to CD3 and BCMA, and Bispecific Binding Proteins Made Therefrom. Applicant: Shanghai EpimAb Biotherapeutics Co., Ltd. Application EP. The sequence listing filed with the application follows.

SEQUENCE LISTING (88 sequences)

SEQ ID NO: 1 - protein, 227 aa, synthetic construct
  REGION 1..227: note = Synthetic
DKTHTCPPCPAPEAAGGPSVFLFPPKPKDTLMISRTPEVTCVVVDVSHEDPEVKFNWYVDGVEVHNAKTKPREEQYNSTYRVVSVLTVLHQDWLNGKEYKCKVSNKALPAPIEKTISKAKGQPREPQVYTLPPSREEMTKNQVSLTCLVKGFYPSDIAVEWESNGQPENNYKTTPPVLDSDGSFFLYSKLTVDKSRWQQGNVFSCSVMHEALHNHYTQKSLSLSPGK

SEQ ID NO: 2 - protein, 17 aa, synthetic construct
  REGION 1..17: note = Synthetic
LSLKEFSELEQSGYYVC

SEQ ID NO: 3 - protein, 16 aa, synthetic construct
  REGION 1..16: note = Synthetic
QDGNEEMGGITQTPYK

SEQ ID NO: 4 - protein, 338 aa, synthetic construct
  REGION 1..338: note = Synthetic
QDGNEEMGGITQTPYKVSISGTTVILTCPQYPGSEILWQHNDKNIGGDEDDKNIGSDEDHLSLKEFSELEQSGYYVCYPRGSKPEDANFYLYLRARVCENCMEMDGSSGSSDKTHTCPPCPAPELLGGPSVFLFPPKPKDTLMISRTPEVTCVVVDVSHEDPEVKFNWYVDGVEVHNAKTKPREEQYNSTYRVVSVLTVLHQDWLNGKEYKCKVSNKALPAPIEKTISKAKGQPREPQVYTLPPCRDELTKNQVSLWCLVKGFYPSDIAVEWESNGQPENNYKTTPPVLDSDGSFFLYSKLTVDKSRWQQGNVFSCSVMHEALHNHYTQKSLSLSPGK

SEQ ID NO: 5 - protein, 327 aa, synthetic construct
  REGION 1..327: note = Synthetic
QSIKGNHLVKVYDYQEDGSVLLTCDAEAKNITWFKDGKMIGFLTEDKKKWNLGSNAKDPRGMYQCKGSQNKSKPLQVYYRMCQNCIELNAATISGSSGSSDKTHTCPPCPAPELLGGPSVFLFPPKPKDTLMISRTPEVTCVVVDVSHEDPEVKFNWYVDGVEVHNAKTKPREEQYNSTYRVVSVLTVLHQDWLNGKEYKCKVSNKALPAPIEKTISKAKGQPREPQVCTLPPSRDELTKNQVSLSCAVKGFYPSDIAVEWESNGQPENNYKTTPPVLDSDGSFFLVSKLTVDKSRWQQGNVFSCSVMHEALHNHYTQKSLSLSPGK

SEQ ID NO: 6 - protein, 119 aa, synthetic construct
  REGION 1..119: note = Synthetic
QVQLQQSGPDLVKPGASVKISCKASGFSFTNYYVHWMKQRPGQGLEWIGWISPGSDNTKYNEKFKGKATLTADTSSTTAYMQLSSLTSEDSAVYYCARDDYGNYYFDYWGRGSTLTVSS

SEQ ID NO: 7 - protein, 112 aa, synthetic construct
  REGION 1..112: note = Synthetic
DIVMSQSPSSLAVSAGEKVTMTCKSSQSLLNSRTRKNYLAWYQQKPGQSPKLLIYWASTRESGVPDRFTGSGSGTDFTLTISSVQAEDLAVYYCKQSYILRTFGGGTKLEIK

SEQ ID NO: 8 - protein, 119 aa, synthetic construct
  REGION 1..119: note = Synthetic
QVQLQQSGPELVKPGASVRISCKASGYTFTNYYIHWVKQRPGQGLEWIGWINLGDVNTKFNEKFKDKATLTADKSSTTAYMQLSSLTSEDSAVYFCARDGYSFYYFDFWGQGTTLTVSS

SEQ ID NO: 9 - protein, 112 aa, synthetic construct
  REGION 1..112: note = Synthetic
DIVMSQSPSSLAVSVGEKVTMSCKASQSLFNSRTRKNYLAWYQQKPGQSPKLLIYWASTRESGVPDRFTGSGSGTDFIFTISSVQAEDLAIYYCIQSHTLRTFGGGTKLEIK

SEQ ID NO: 10 - protein, 119 aa, synthetic construct
  REGION 1..119: note = Synthetic
EVQLVQSGAEVKKPGASVKVSCKASGYTFTNYYVHWVRQAPGQGLEWMGWISPGSDNTKYNEKFKGRVTMTRDTSISTAYMELSRLRSDDTAVYYCARDDYGNYYFDYWGQGTTVTVSS

SEQ ID NO: 11 - protein, 119 aa, synthetic construct
  REGION 1..119: note = Synthetic
EVQLVQSGAEVKKPGASVKVSCKASGYTFTNYYVHWVRQAPGQGLEWMGWISPGSDNTKYNEKFKGRVTLTADTSISTAYMELSRLRSDDTAVYYCARDDYGNYYFDYWGQGTTVTVSS

SEQ ID NO: 12 - protein, 119 aa, synthetic construct
  REGION 1..119: note = Synthetic
EVQLVQSGAEVKKPGASVKVSCKASGYTFTNYYVHWVRQAPGQGLEWIGWISPGSDNTKYNEKFKGRVTLTADTSISTAYMELSRLRSDDTAVYYCARDDYGNYYFDYWGQGTTVTVSS

SEQ ID NO: 13 - protein, 119 aa, synthetic construct
  REGION 1..119: note = Synthetic
EVQLVQSGAEVKKPGASVKVSCKASGYTFTNYYVHWVRQAPGQGLEWIGWISPGSDNTKYNEKFKGKATLTADTSISTAYMELSRLRSDDTAVYYCARDDYGNYYFDYWGQGTTVTVSS

SEQ ID NO: 14 - protein, 119 aa, synthetic construct
  REGION 1..119: note = Synthetic
EVQLVQSGAEVKKPGASVKVSCKASGYTFTNYYVHWMRQAPGQGLEWIGWISPGSDNTKYNEKFKGKATLTADTSISTAYMELSRLRSDDTAVYYCARDDYGNYYFDYWGQGTTVTVSS

SEQ ID NO: 15 - protein, 119 aa, synthetic construct
  REGION 1..119: note = Synthetic
EVQLVQSGAEVKKPGASVKVSCKASGYTFTNYYVHWMRQAPGQGLEWIGWISPGSDNTKYNEKFKGRVTLTADTSISTAYMELSRLRSDDTAVYYCARDDYGNYYFDYWGQGTTVTVSS

SEQ ID NO: 16 - protein, 119 aa, synthetic construct
  REGION 1..119: note = Synthetic
EVQLVQSGAEVKKPGASVKVSCKASGFSFTNYYVHWMRQAPGQGLEWIGWISPGSDNTKYNEKFKGKATLTADTSISTAYMELSRLRSDDTAVYYCARDDYGNYYFDYWGQGTTVTVSS

SEQ ID NO: 17 - protein, 119 aa, synthetic construct
  REGION 1..119: note = Synthetic
EVQLVQSGAEVKKPGASVKVSCKASGFSFTNYYVHWMRQAPGQGLEWIGWISPGSDNTKYNEKFKGRVTLTADTSISTAYMELSRLRSDDTAVYYCARDDYGNYYFDYWGQGTTVTVSS

SEQ ID NO: 18 - protein, 119 aa, synthetic construct
  REGION 1..119: note = Synthetic
EVQLVQSGAEVKKPGASVKVSCKASGFSFTNYYVHWMRQAPGQGLEWMGWISPGSDNTKYNEKFKGRVTMTRDTSISTAYMELSRLRSDDTAVYYCARDDYGNYYFDYWGQGTTVTVSS

SEQ ID NO: 19 - protein, 119 aa, synthetic construct
  REGION 1..119: note = Synthetic
EVQLVQSGAEVKKPGASVKVSCKASGFSFTNYYVHWMKQAPGQGLEWIGWISPGSDNTKYNEKFKGKATLTADTSITTAYMELSRLRSDDTAVYYCARDDYGNYYFDYWGQGTTVTVSS

SEQ ID NO: 20 - protein, 112 aa, synthetic construct
  REGION 1..112: note = Synthetic
DIVMTQSPDSLAVSLGERATINCKSSQSLLNSRTRKNYLAWYQQKPGQPPKLLIYWASTRESGVPDRFSGSGSGTDFTLTISSLQAEDVAVYYCKQSYILRTFGGGTKVEIK

SEQ ID NO: 21 - protein, 112 aa, synthetic construct
  REGION 1..112: note = Synthetic
DIVMSQSPDSLAVSLGERATITCKSSQSLLNSRTRKNYLAWYQQKPGQPPKLLIYWASTRESGVPDRFSGSGSGTDFTLTISSLQAEDVAVYYCKQSYILRTFGGGTKVEIK

SEQ ID NO: 22 - protein, 112 aa, synthetic construct
  REGION 1..112: note = Synthetic
DIVMTQSPDSLAVSLGERATINCKSSQSLLQSRTRKNYLAWYQQKPGQPPKLLIYWASTRESGVPDRFSGSGSGTDFTLTISSLQAEDVAVYYCKQSYILRTFGGGTKVEIK

SEQ ID NO: 23 - protein, 112 aa, synthetic construct
  REGION 1..112: note = Synthetic
DIVMSQSPDSLAVSLGERATITCKSSQSLLQSRTRKNYLAWYQQKPGQPPKLLIYWASTRESGVPDRFSGSGSGTDFTLTISSLQAEDVAVYYCKQSYILRTFGGGTKVEIK

SEQ ID NO: 24 - protein, 112 aa, synthetic construct
  REGION 1..112: note = Synthetic
DIVMTQSPDSLAVSLGERATINCKSSQSLLNTRTRKNYLAWYQQKPGQPPKLLIYWASTRESGVPDRFSGSGSGTDFTLTISSLQAEDVAVYYCKQSYILRTFGGGTKVEIK

SEQ ID NO: 25 - protein, 112 aa, synthetic construct
  REGION 1..112: note = Synthetic
DIVMTQSPDSLAVSLGERATINCKSSQSLLNARTRKNYLAWYQQKPGQPPKLLIYWASTRESGVPDRFSGSGSGTDFTLTISSLQAEDVAVYYCKQSYILRTFGGGTKVEIK

SEQ ID NO: 26 - protein, 330 aa, synthetic construct
  REGION 1..330: note = Synthetic
ASTKGPSVFPLAPSSKSTSGGTAALGCLVKDYFPEPVTVSWNSGALTSGVHTFPAVLQSSGLYSLSSVVTVPSSSLGTQTYICNVNHKPSNTKVDKKVEPKSCDKTHTCPPCPAPEAAGGPSVFLFPPKPKDTLMISRTPEVTCVVVDVSHEDPEVKFNWYVDGVEVHNAKTKPREEQYNSTYRVVSVLTVLHQDWLNGKEYKCKVSNKALPAPIEKTISKAKGQPREPQVYTLPPSREEMTKNQVSLTCLVKGFYPSDIAVEWESNGQPENNYKTTPPVLDSDGSFFLYSKLTVDKSRWQQGNVFSCSVMHEALHNHYTQKSLSLSPGK

SEQ ID NO: 27 - protein, 107 aa, synthetic construct [sequence omitted]

SEQ ID NO: 28 - protein, 291 aa, synthetic construct
  REGION 1..291: note = Synthetic
MLQMAGQCSQNEYFDSLLHACIPCQLRCSSNTPPLTCQRYCNASVTNSVKGTNAIEGRMDPKSCDKTHTCPPCPAPELLGGPSVFLFPPKPKDTLMISRTPEVTCVVVDVSHEDPEVKFNWYVDGVEVHNAKTKPREEQYNSTYRVVSVLTVLHQDWLNGKEYKCKVSNKALPAPIEKTISKAKGQPREPQVYTLPPSREEMTKNQVSLTCLVKGFYPSDIAVEWESNGQPENNYKTTPPVLDSDGSFFLYSKLTVDKSRWQQGNVFSCSVMHEALHNHYTQKSLSLSPGK

SEQ ID NO: 29 - protein, 121 aa, synthetic construct
  REGION 1..121: note = Synthetic
QIQLVQSGPELKKPGETVKISCKASGYSFTNYGLNWVKQAPGKGLKWMGWINTYSGHPTYVDDFKGRFAFSLETSASTAYLQINKLKNEDTSTYFCVREKDDGYRLGLDYWGQGTSVTVSS

SEQ ID NO: 30 - protein, 106 aa, synthetic construct
  REGION 1..106: note = Synthetic
QIVLTQSPAIMSASPGEKVTMTCSASSSVSYMYWYQQRPGSSPRLWIYDTSNLVSGVPARFSGSRSGTSYSLTISGMEAEDAATYYCLQYSGYPYTFGGGTKLEIK

SEQ ID NO: 31 - protein, 121 aa, synthetic construct
  REGION 1..121: note = Synthetic
EVQLQQSGTVLARPGASVRMSCKASGYIFPNFWMHWVKQRPGQGLDWIGAFYPGNDDTYYNQKFKGKAKLTAVTSASTAYMELSSLTSEDSAVYYCARSGYYGSSDAMDYWGQGTSVTVSS

SEQ ID NO: 32 - protein, 107 aa, synthetic construct
  REGION 1..107: note = Synthetic
DIQMTQSPASLSASVGETVTVTCGASENIYGALNWYQRKQGKSPQLLIYGATNLADGISSRFSGSGSGRQFSLKISSLLPDDVATYFCQSVLTTPWTFGGGTKLEIK

SEQ ID NO: 33 - protein, 121 aa, synthetic construct
  REGION 1..121: note = Synthetic
EVQLVQSGAEVKKPGASVKVSCKASGYTFTNFWMHWVRQAPGQRLEWMGAFYPGNDDTYYNQKFKGRVTITRDTSASTAYMELSSLRSEDMAVYYCARSGYYGSSDAMDYWGQGTTVTVSS

SEQ ID NO: 34 - protein, 121 aa, synthetic construct
  REGION 1..121: note = Synthetic
EVQLVQSGAEVKKPGASVKVSCKASGYTFTNFWMHWVRQAPGQRLEWMGAFYPGNDDTYYNQKFKGRVTITADTSASTAYMELSSLRSEDMAVYYCARSGYYGSSDAMDYWGQGTTVTVSS

SEQ ID NO: 35 - protein, 121 aa, synthetic construct
  REGION 1..121: note = Synthetic
EVQLVQSGAEVKKPGASVKVSCKASGYTFTNFWMHWVRQAPGQRLEWIGAFYPGNDDTYYNQKFKGKATLTADTSASTAYMELSSLRSEDMAVYYCARSGYYGSSDAMDYWGQGTTVTVSS

SEQ ID NO: 36 - protein, 121 aa, synthetic construct
  REGION 1..121: note = Synthetic
EVQLVQSGAEVKKPGASVKVSCKASGYTFPNFWMHWVRQAPGQRLEWIGAFYPGNDDTYYNQKFKGKATLTADTSASTAYMELSSLRSEDMAVYYCARSGYYGSSDAMDYWGQGTTVTVSS

SEQ ID NO: 37 - protein, 121 aa, synthetic construct
  REGION 1..121: note = Synthetic
EVQLVQSGAEVKKPGASVKVSCKASGYTFPNFWMHWVRQAPGQRLEWMGAFYPGNDDTYYNQKFKGRVTITRDTSASTAYMELSSLRSEDMAVYYCARSGYYGSSDAMDYWGQGTTVTVSS

SEQ ID NO: 38 - protein, 107 aa, synthetic construct
  REGION 1..107: note = Synthetic
DIQMTQSPSSLSASVGDRVTITCGASENIYGALNWYQQKPGKAPKLLIYGATNLADGVPSRFSGSGSGTDFTLTISSLQPEDFATYYCQSVLTTPWTFGQGTKLEIK

SEQ ID NO: 39 - protein, 107 aa, synthetic construct
  REGION 1..107: note = Synthetic
DIQMTQSPSSLSASVGDRVTITCGASENIYGALNWYQQKPGKAPKLLIYGATNLADGIPSRFSGSGSGRDFTLTISSLQPEDFATYYCQSVLTTPWTFGQGTKLEIK

SEQ ID NO: 40 - protein, 107 aa, synthetic construct
  REGION 1..107: note = Synthetic
DIQMTQSPSSLSASVGDRVTITCGASENIYGALNWYQQKPGKAPKLLIYGATNLAAGVPSRFSGSGSGTDFTLTISSLQPEDFATYYCQSVLTTPWTFGQGTKLEIK

SEQ ID NO: 41 - protein, 107 aa, synthetic construct
  REGION 1..107: note = Synthetic
DIQMTQSPSSLSASVGDRVTITCGASENIYGALNWYQQKPGKAPKLLIYGATNLAEGVPSRFSGSGSGTDFTLTISSLQPEDFATYYCQSVLTTPWTFGQGTKLEIK

SEQ ID NO: 42 - protein, 107 aa, synthetic construct
  REGION 1..107: note = Synthetic
DIQMTQSPSSLSASVGDRVTITCGASENIYGALNWYQQKPGKAPKLLIYGATNLASGVPSRFSGSGSGTDFTLTISSLQPEDFATYYCQSVLTTPWTFGQGTKLEIK

SEQ ID NO: 43 - protein, 107 aa, synthetic construct
  REGION 1..107: note = Synthetic
DIQMTQSPSSLSASVGDRVTITCGASENIYGALNWYQQKPGKAPKLLIYGATNLATGVPSRFSGSGSGTDFTLTISSLQPEDFATYYCQSVLTTPWTFGQGTKLEIK

SEQ ID NO: 44 - protein, 107 aa, synthetic construct
  REGION 1..107: note = Synthetic
DIQMTQSPSSLSASVGDRVTITCGASENIYGALNWYQQKPGKAPKLLIYGATNLADAVPSRFSGSGSGTDFTLTISSLQPEDFATYYCQSVLTTPWTFGQGTKLEIK

SEQ ID NO: 45 - protein, 107 aa, synthetic construct
  REGION 1..107: note = Synthetic
DIQMTQSPSSLSASVGDRVTITCGASENIYGALNWYQQKPGKAPKLLIYGATNLAAGIPSRFSGSGSGRDFTLTISSLQPEDFATYYCQSVLTTPWTFGQGTKLEIK

SEQ ID NO: 46 - protein, 107 aa, synthetic construct
  REGION 1..107: note = Synthetic
DIQMTQSPSSLSASVGDRVTITCGASENIYGALNWYQQKPGKAPKLLIYGATNLAEGIPSRFSGSGSGRDFTLTISSLQPEDFATYYCQSVLTTPWTFGQGTKLEIK

SEQ ID NO: 47 - protein, 107 aa, synthetic construct
  REGION 1..107: note = Synthetic
DIQMTQSPSSLSASVGDRVTITCGASENIYGALNWYQQKPGKAPKLLIYGATNLASGIPSRFSGSGSGRDFTLTISSLQPEDFATYYCQSVLTTPWTFGQGTKLEIK

SEQ ID NO: 48 - protein, 107 aa, synthetic construct
  REGION 1..107: note = Synthetic
DIQMTQSPSSLSASVGDRVTITCGASENIYGALNWYQQKPGKAPKLLIYGATNLATGIPSRFSGSGSGRDFTLTISSLQPEDFATYYCQSVLTTPWTFGQGTKLEIK

SEQ ID NO: 49 - protein, 107 aa, synthetic construct
  REGION 1..107: note = Synthetic
DIQMTQSPSSLSASVGDRVTITCGASENIYGALNWYQQKPGKAPKLLIYGATNLADAIPSRFSGSGSGRDFTLTISSLQPEDFATYYCQSVLTTPWTFGQGTKLEIK

SEQ ID NO: 50 - protein, 663 aa, synthetic construct
  REGION 1..663: note = Synthetic
DIQMTQSPSSLSASVGDRVTITCGASENIYGALNWYQQKPGKAPKLLIYGATNLAAGVPSRFSGSGSGTDFTLTISSLQPEDFATYYCQSVLTTPWTFGQGTKLEIKRTVAAPSVFIFPPSDEQLKSGTASVVCLLNNFYPREAKVQWKVDNALQSGNSQESVTEQDSKDSTYSLSSTLTLSKADYEKHKVYACEVTHQGLSSPVTKSFNRGECEVQLVQSGAEVKKPGASVKVSCKASGFSFTNYYVHWMRQAPGQGLEWMGWISPGSDNTKYNEKFKGRVTMTRDTSISTAYMELSRLRSDDTAVYYCARDDYGNYYFDYWGQGTTVTVSSASTKGPSVFPLAPSSKSTSGGTAALGCLVKDYFPEPVTVSWNSGALTSGVHTFPAVLQSSGLYSLSSVVTVPSSSLGTQTYICNVNHKPSNTKVDKKVEPKSCDKTHTCPPCPAPEAAGGPSVFLFPPKPKDTLMISRTPEVTCVVVDVSHEDPEVKFNWYVDGVEVHNAKTKPREEQYNSTYRVVSVLTVLHQDWLNGKEYKCKVSNKALPAPIEKTISKAKGQPREPQVYTLPPSREEMTKNQVSLTCLVKGFYPSDIAVEWESNGQPENNYKTTPPVLDSDGSFFLYSKLTVDKSRWQQGNVFSCSVMHEALHNHYTQKSLSLSPGK

SEQ ID NO: 51 - protein, 224 aa, synthetic construct
  REGION 1..224: note = Synthetic
EVQLVQSGAEVKKPGASVKVSCKASGYTFPNFWMHWVRQAPGQRLEWIGAFYPGNDDTYYNQKFKGKATLTADTSASTAYMELSSLRSEDMAVYYCARSGYYGSSDAMDYWGQGTTVTVSSASTKGPSVFPLAPSSKSTSGGTAALGCLVKDYFPEPVTVSWNSGALTSGVHTFPAVLQSSGLYSLSSVVTVPSSSLGTQTYICNVNHKPSNTKVDKKVEPKSC

SEQ ID NO: 52 - protein, 219 aa, synthetic construct
  REGION 1..219: note = Synthetic
DIVMTQSPDSLAVSLGERATINCKSSQSLLNARTRKNYLAWYQQKPGQPPKLLIYWASTRESGVPDRFSGSGSGTDFTLTISSLQAEDVAVYYCKQSYILRTFGGGTKVEIKRTVAAPSVFIFPPSDEQLKSGTASVVCLLNNFYPREAKVQWKVDNALQSGNSQESVTEQDSKDSTYSLSSTLTLSKADYEKHKVYACEVTHQGLSSPVTKSFNRGEC

SEQ ID NO: 53 - protein, 663 aa, synthetic construct
  REGION 1..663: note = Synthetic
DIQMTQSPSSLSASVGDRVTITCGASENIYGALNWYQQKPGKAPKLLIYGATNLATGIPSRFSGSGSGRDFTLTISSLQPEDFATYYCQSVLTTPWTFGQGTKLEIKRTVAAPSVFIFPPSDEQLKSGTASVVCLLNNFYPREAKVQWKVDNALQSGNSQESVTEQDSKDSTYSLSSTLTLSKADYEKHKVYACEVTHQGLSSPVTKSFNRGECEVQLVQSGAEVKKPGASVKVSCKASGFSFTNYYVHWMRQAPGQGLEWMGWISPGSDNTKYNEKFKGRVTMTRDTSISTAYMELSRLRSDDTAVYYCARDDYGNYYFDYWGQGTTVTVSSASTKGPSVFPLAPSSKSTSGGTAALGCLVKDYFPEPVTVSWNSGALTSGVHTFPAVLQSSGLYSLSSVVTVPSSSLGTQTYICNVNHKPSNTKVDKKVEPKSCDKTHTCPPCPAPEAAGGPSVFLFPPKPKDTLMISRTPEVTCVVVDVSHEDPEVKFNWYVDGVEVHNAKTKPREEQYNSTYRVVSVLTVLHQDWLNGKEYKCKVSNKALPAPIEKTISKAKGQPREPQVYTLPPSREEMTKNQVSLTCLVKGFYPSDIAVEWESNGQPENNYKTTPPVLDSDGSFFLYSKLTVDKSRWQQGNVFSCSVMHEALHNHYTQKSLSLSPGK

SEQ ID NO: 54 - protein, 224 aa, synthetic construct
  REGION 1..224: note = Synthetic
EVQLVQSGAEVKKPGASVKVSCKASGYTFTNFWMHWVRQAPGQRLEWMGAFYPGNDDTYYNQKFKGRVTITADTSASTAYMELSSLRSEDMAVYYCARSGYYGSSDAMDYWGQGTTVTVSSASTKGPSVFPLAPSSKSTSGGTAALGCLVKDYFPEPVTVSWNSGALTSGVHTFPAVLQSSGLYSLSSVVTVPSSSLGTQTYICNVNHKPSNTKVDKKVEPKSC

SEQ ID NO: 55 - protein, 219 aa, synthetic construct; identical to SEQ ID NO: 52
  REGION 1..219: note = Synthetic

SEQ ID NO: 56 - protein, 5 aa, synthetic construct
  REGION 1..5: note = Synthetic
NYYVH

SEQ ID NO: 57 - protein, 17 aa, synthetic construct
  REGION 1..17: note = Synthetic
WISPGSDNTKYNEKFKG

SEQ ID NO: 58 - protein, 10 aa, synthetic construct
  REGION 1..10: note = Synthetic
DDYGNYYFDY

SEQ ID NO: 59 - protein, 17 aa, synthetic construct
  REGION 1..17: note = Synthetic
KSSQSLLNSRTRKNYLA

SEQ ID NO: 60 - protein, 7 aa, synthetic construct
  REGION 1..7: note = Synthetic
WASTRES

SEQ ID NO: 61 - protein, 8 aa, synthetic construct
  REGION 1..8: note = Synthetic
KQSYILRT

SEQ ID NO: 62 - protein, 5 aa, synthetic construct
  REGION 1..5: note = Synthetic
NYYIH

SEQ ID NO: 63 - protein, 17 aa, synthetic construct
  REGION 1..17: note = Synthetic
WINLGDVNTKFNEKFKD

SEQ ID NO: 64 - protein, 10 aa, synthetic construct
  REGION 1..10: note = Synthetic
DGYSFYYFDF

SEQ ID NO: 65 - protein, 17 aa, synthetic construct
  REGION 1..17: note = Synthetic
KASQSLFNSRTRKNYLA

SEQ ID NO: 66 - protein, 7 aa, synthetic construct
  REGION 1..7: note = Synthetic
WASTRES

SEQ ID NO: 67 - protein, 8 aa, synthetic construct
  REGION 1..8: note = Synthetic
IQSHTLRT

SEQ ID NO: 68 - protein, 5 aa, synthetic construct
  REGION 1..5: note = Synthetic
NYGLN

SEQ ID NO: 69 - protein, 17 aa, synthetic construct
  REGION 1..17: note = Synthetic
WINTYSGHPTYVDDFKG

SEQ ID NO: 70 - protein, 12 aa, synthetic construct
  REGION 1..12: note = Synthetic
EKDDGYRLGLDY

SEQ ID NO: 71 - protein, 10 aa, synthetic construct
  REGION 1..10: note = Synthetic
SASSSVSYMY

SEQ ID NO: 72 - protein, 7 aa, synthetic construct
  REGION 1..7: note = Synthetic
DTSNLVS

SEQ ID NO: 73 - protein, 9 aa, synthetic construct
  REGION 1..9: note = Synthetic
LQYSGYPYT

SEQ ID NO: 74 - protein, 5 aa, synthetic construct
  REGION 1..5: note = Synthetic
NFWMH

SEQ ID NO: 75 - protein, 16 aa, synthetic construct
  REGION 1..16: note = Synthetic
AFYPGNDDTYYNQKFK

SEQ ID NO: 76 - protein, 12 aa, synthetic construct
  REGION 1..12: note = Synthetic
SGYYGSSDAMDY

SEQ ID NO: 77 - protein, 11 aa, synthetic construct
  REGION 1..11: note = Synthetic
GASENIYGALN

SEQ ID NO: 78 - protein, 7 aa, synthetic construct
  REGION 1..7: note = Synthetic
GATNLAD

SEQ ID NO: 79 - protein, 9 aa, synthetic construct
  REGION 1..9: note = Synthetic
QSVLTTPWT

SEQ ID NO: 80 - protein, 663 aa, synthetic construct
  REGION 1..663: note = Synthetic
DIQMTQSPSSLSASVGDRVTITCGASENIYGALNWYQQKPGKAPKLLIYGATNLATGIPSRFSGSGSGRDFTLTISSLQPEDFATYYCQSVLTTPWTFGQGTKLEIKRTVAAPSVFIFPPSDEQLKSGTASVVCLLNNFYPREAKVQWKVDNALQSGNSQESVTEQDSKDSTYSLSSTLTLSKADYEKHKVYACEVTHQGLSSPVTKSFNRGECEVQLVQSGAEVKKPGASVKVSCKASGFSFTNYYVHWMRQAPGQGLEWIGWISPGSDNTKYNEKFKGRVTLTADTSISTAYMELSRLRSDDTAVYYCARDDYGNYYFDYWGQGTTVTVSSASTKGPSVFPLAPSSKSTSGGTAALGCLVKDYFPEPVTVSWNSGALTSGVHTFPAVLQSSGLYSLSSVVTVPSSSLGTQTYICNVNHKPSNTKVDKKVEPKSCDKTHTCPPCPAPEAAGGPSVFLFPPKPKDTLMISRTPEVTCVVVDVSHEDPEVKFNWYVDGVEVHNAKTKPREEQYNSTYRVVSVLTVLHQDWLNGKEYKCKVSNKALPAPIEKTISKAKGQPREPQVYTLPPSREEMTKNQVSLTCLVKGFYPSDIAVEWESNGQPENNYKTTPPVLDSDGSFFLYSKLTVDKSRWQQGNVFSCSVMHEALHNHYTQKSLSLSPGK

SEQ ID NO: 81 - protein, 224 aa, synthetic construct; identical to SEQ ID NO: 54
  REGION 1..224: note = Synthetic

SEQ ID NO: 82 - protein, 219 aa, synthetic construct; identical to SEQ ID NO: 52
  REGION 1..219: note = Synthetic

SEQ ID NO: 83 - protein, 670 aa, synthetic construct
  REGION 1..670: note = Synthetic
DIVMTQSPDSLAVSLGERATINCKSSQSLLNARTRKNYLAWYQQKPGQPPKLLIYWASTRESGVPDRFSGSGSGTDFTLTISSLQAEDVAVYYCKQSYILRTFGGGTKVEIKRTVAAPSVFIFPPSDEQLKSGTASVVCLLNNFYPREAKVQWKVDNALQSGNSQESVTEQDSKDSTYSLSSTLTLSKADYEKHKVYACEVTHQGLSSPVTKSFNRGECEVQLVQSGAEVKKPGASVKVSCKASGYTFTNFWMHWVRQAPGQRLEWMGAFYPGNDDTYYNQKFKGRVTITADTSASTAYMELSSLRSEDMAVYYCARSGYYGSSDAMDYWGQGTTVTVSSASTKGPSVFPLAPSSKSTSGGTAALGCLVKDYFPEPVTVSWNSGALTSGVHTFPAVLQSSGLYSLSSVVTVPSSSLGTQTYICNVNHKPSNTKVDKKVEPKSCDKTHTCPPCPAPEAAGGPSVFLFPPKPKDTLMISRTPEVTCVVVDVSHEDPEVKFNWYVDGVEVHNAKTKPREEQYNSTYRVVSVLTVLHQDWLNGKEYKCKVSNKALPAPIEKTISKAKGQPREPQVYTLPPSREEMTKNQVSLTCLVKGFYPSDIAVEWESNGQPENNYKTTPPVLDSDGSFFLYSKLTVDKSRWQQGNVFSCSVMHEALHNHYTQKSLSLSPGK

SEQ ID NO: 84 - protein, 222 aa, synthetic construct
  REGION 1..222: note = Synthetic
EVQLVQSGAEVKKPGASVKVSCKASGFSFTNYYVHWMRQAPGQGLEWMGWISPGSDNTKYNEKFKGRVTMTRDTSISTAYMELSRLRSDDTAVYYCARDDYGNYYFDYWGQGTTVTVSSASTKGPSVFPLAPSSKSTSGGTAALGCLVKDYFPEPVTVSWNSGALTSGVHTFPAVLQSSGLYSLSSVVTVPSSSLGTQTYICNVNHKPSNTKVDKKVEPKSC

SEQ ID NO: 85 - protein, 214 aa, synthetic construct
  REGION 1..214: note = Synthetic
DIQMTQSPSSLSASVGDRVTITCGASENIYGALNWYQQKPGKAPKLLIYGATNLATGIPSRFSGSGSGRDFTLTISSLQPEDFATYYCQSVLTTPWTFGQGTKLEIKRTVAAPSVFIFPPSDEQLKSGTASVVCLLNNFYPREAKVQWKVDNALQSGNSQESVTEQDSKDSTYSLSSTLTLSKADYEKHKVYACEVTHQGLSSPVTKSFNRGEC

SEQ ID NO: 86 - protein, 670 aa, synthetic construct; identical to SEQ ID NO: 83
  REGION 1..670: note = Synthetic

SEQ ID NO: 87 - protein, 222 aa, synthetic construct
  REGION 1..222: note = Synthetic
EVQLVQSGAEVKKPGASVKVSCKASGFSFTNYYVHWMRQAPGQGLEWIGWISPGSDNTKYNEKFKGRVTLTADTSISTAYMELSRLRSDDTAVYYCARDDYGNYYFDYWGQGTTVTVSSASTKGPSVFPLAPSSKSTSGGTAALGCLVKDYFPEPVTVSWNSGALTSGVHTFPAVLQSSGLYSLSSVVTVPSSSLGTQTYICNVNHKPSNTKVDKKVEPKSC

SEQ ID NO: 88 - protein, 214 aa, synthetic construct; identical to SEQ ID NO: 85
  REGION 1..214: note = Synthetic